European Patent Application EP 4 501 354 A1, published February 5, 2025. Title: Compositions or methods for suppressing fibrosis. Applicant: Pharma Foods International Co., Ltd. Application WO. The sequence listing filed with the application follows.

SEQUENCE LISTING (54 sequences)

SEQ ID NO: 1 - protein, 665 aa, Homo sapiens
MLRERTVRLQYGSRVEAVYVLGTYLWTDVYSAAPAGAQTFSLKHSEHVWVEVVRDGEAEEVATNGKQRWLLSPSTTLRVTMSQASTEASSDKVTVNYYDEEGSIPIDQAGLFLTAIEISLDVDADRDGVVEKNNPKKASWTWGPEGQGAILLVNCDRETPWLPKEDCRDEKVYSKEDLKDMSQMILRTKGPDRLPAGYEIVLYISMSDSDKVGVFYVENPFFGQRYIHILGRRKLYHVVKYTGGSAELLFFVEGLCFPDEGFSGLVSIHVSLLEYMAQDIPLTPIFTDTVIFRIAPWIMTPNILPPVSVFVCCMKDNYLFLKEVKNLVEKTNCELKVCFQYLNRGDRWIQDEIEFGYIEAPHKGFPVVLDSPRDGNLKDFPVKELLGPDFGYVTREPLFESVTSLDSFGNLEVSPPVTVNGKTYPLGRILIGSSFPLSGGRRMTKVVRDFLKAQQVQAPVELYSDWLTVGHVDEFMSFVPIPGTKKFLLLMASTSACYKLFREKQKDGHGEAIMFKGLGGMSSKRITINKILSNESLVQENLYFQRCLDWNRDILKKELGLTEQDIIDLPALFKMDEDHRARAFFPNMVNMIVLDKDLGIPKPFGPQVEEECCLEMHVRGLLEPLGLECTFIDDISAYHKFLGEVHCGTNVRRKPFTFKWWHMVP

SEQ ID NO: 2 - protein, 17 aa, synthetic construct
  REGION 1..17: note = peptide antigen
YLNRGDRWIQDEIEFGY

SEQ ID NO: 3 - protein, 5 aa, Gallus gallus
SYAMY

SEQ ID NO: 4 - protein, 17 aa, Gallus gallus
GISSSGRYTGYAPAVKG

SEQ ID NO: 5 - protein, 14 aa, Gallus gallus
DVYDSWTYANRIDA

SEQ ID NO: 6 - protein, 10 aa, Gallus gallus
SGGGRRGYYG

SEQ ID NO: 7 - protein, 7 aa, Gallus gallus
NNDERPS

SEQ ID NO: 8 - protein, 11 aa, Gallus gallus
GSGDTTTDSGI

SEQ ID NO: 9 - protein, 5 aa, Gallus gallus
DYGMG

SEQ ID NO: 10 - protein, 17 aa, Gallus gallus
AISNRGSHTYYGAAVKG

SEQ ID NO: 11 - protein, 21 aa, Gallus gallus
DAGTCISSYGFSCVSAASIDA

SEQ ID NO: 12 - protein, 14 aa, Gallus gallus
SGGSGSYGGSYYYG

SEQ ID NO: 13 - protein, 7 aa, Gallus gallus
DNTNRPS

SEQ ID NO: 14 - protein, 11 aa, Gallus gallus
GSIDSISDADI

SEQ ID NO: 15 - protein, 5 aa, Gallus gallus
RYAIQ

SEQ ID NO: 16 - protein, 16 aa, Gallus gallus
VINSGGRTLYAPAVKG

SEQ ID NO: 17 - protein, 9 aa, Gallus gallus
GGYAYGIET

SEQ ID NO: 18 - protein, 8 aa, Gallus gallus
SGSRYDYG

SEQ ID NO: 19 - protein, 7 aa, Gallus gallus
YNNKRPS

SEQ ID NO: 20 - protein, 9 aa, Gallus gallus
GSTDTSNDI

SEQ ID NO: 21 - protein, 123 aa, Gallus gallus
AVTLDESGGGLQTPGGGLSLVCKASGFTFRSYAMYWVRQAPGKGLEWLAGISSSGRYTGYAPAVKGRATISRDNGQSTVRLQLSNLRAEDAGTYYCAKDVYDSWTYANRIDAWGHGTEVIVSS

SEQ ID NO: 22 - protein, 106 aa, Gallus gallus
ALTQPSSVSANPGETVKITCSGGGRRGYYGWYQQKSPGSAPVTVIYNNDERPSNIPSRFSGFKSGSTATLTITGVQAEDEAVYYCGSGDTTTDSGIFGAGTTLTVL

SEQ ID NO: 23 - protein, 130 aa, Gallus gallus
AVTLDESGGGLQTPGRALSLVCKASGFTFSDYGMGWMRQAPGKGLEWVGAISNRGSHTYYGAAVKGRATISRDNGQSTVRLQLNNLRAEDTGTYYCAKDAGTCISSYGFSCVSAASIDAWGHGTEVIVSS

SEQ ID NO: 24 - protein, 110 aa, Gallus gallus
ALTQPSSVSANLGGTVKITCSGGSGSYGGSYYYGWYQQKAPGSAPVTLIYDNTNRPSNIPSRFSGSKSGSTATLTITGVQADDEAVYFCGSIDSISDADIFGAGTTLTVL

SEQ ID NO: 25 - protein, 117 aa, Gallus gallus
AVTLDESGGGLQTPGGALSLVCKASGFTFTRYAIQWVRQAPGKGLEWVGVINSGGRTLYAPAVKGRATISRDNGQSTVRLQLNNLRAEDTAIYYCVRGGYAYGIETWGHGTEVIVSS

SEQ ID NO: 26 - protein, 102 aa, Gallus gallus
ALTQPSSVSANPGETVKITCSGSRYDYGWYQQKSPGSAPVTLIYYNNKRPSDIPSRFSGSKSGSTHTLTITGVQADDEAVYFCGSTDTSNDIFGAGTTLTVL

SEQ ID NO: 27 - protein, 330 aa, Homo sapiens [sequence omitted]

SEQ ID NO: 28 - protein, 105 aa, Homo sapiens
GQPKAAPSVTLFPPSSEELQANKATLVCLISDFYPGAVTVAWKADSSPVKAGVETTTPSKQSNNKYAASSYLSLTPEQWKSHRSYSCQVTHEGSTVEKTVAPTEC

SEQ ID NO: 29 - DNA, 15 bp, Gallus gallus
  source 1..15: mol_type = genomic DNA
agttacgccatgtac

SEQ ID NO: 30 - DNA, 51 bp, Gallus gallus
  source 1..51: mol_type = genomic DNA
gggattagtagtagtggtagatacacaggctacgcgccggcggtgaagggc

SEQ ID NO: 31 - DNA, 42 bp, Gallus gallus
  source 1..42: mol_type = genomic DNA
gatgtttacgattcttggacttacgctaatcgtatcgacgca

SEQ ID NO: 32 - DNA, 30 bp, Gallus gallus
  source 1..30: mol_type = genomic DNA
tccgggggtggtaggcgcggttactatggc

SEQ ID NO: 33 - DNA, 21 bp, Gallus gallus
  source 1..21: mol_type = genomic DNA
aacaacgacgagagaccctca

SEQ ID NO: 34 - DNA, 33 bp, Gallus gallus
  source 1..33: mol_type = genomic DNA
gggagtggagacaccactacggatagtggtata

SEQ ID NO: 35 - DNA, 15 bp, Gallus gallus
  source 1..15: mol_type = genomic DNA
gattatggcatgggt

SEQ ID NO: 36 - DNA, 51 bp, Gallus gallus
  source 1..51: mol_type = genomic DNA
gctattagcaacagaggtagtcacacatactacggggcggcggtgaagggc

SEQ ID NO: 37 - DNA, 63 bp, Gallus gallus
  source 1..63: mol_type = genomic DNA
gatgctggtacctgtatttccagttacggtttcagttgtgtatctgctgctagcatcgacgca

SEQ ID NO: 38 - DNA, 42 bp, Gallus gallus
  source 1..42: mol_type = genomic DNA
tccgggggtagtggcagctatggtggaagttactattatggc

SEQ ID NO: 39 - DNA, 21 bp, Gallus gallus
  source 1..21: mol_type = genomic DNA
gacaacaccaacagaccctcg

SEQ ID NO: 40 - DNA, 33 bp, Gallus gallus
  source 1..33: mol_type = genomic DNA
gggagcatagacagcatcagtgatgctgatata

SEQ ID NO: 41 - DNA, 15 bp, Gallus gallus
  source 1..15: mol_type = genomic DNA
cgttacgccatacag

SEQ ID NO: 42 - DNA, 48 bp, Gallus gallus
  source 1..48: mol_type = genomic DNA
gttattaacagtggtggtcgcacactctacgcgccggcggtgaagggc

SEQ ID NO: 43 - DNA, 27 bp, Gallus gallus
  source 1..27: mol_type = genomic DNA
ggtggttatgcttatggcatcgagaca

SEQ ID NO: 44 - DNA, 24 bp, Gallus gallus
  source 1..24: mol_type = genomic DNA
tccgggagtaggtatgattatggc

SEQ ID NO: 45 - DNA, 21 bp, Gallus gallus
  source 1..21: mol_type = genomic DNA
tacaacaacaagagaccctcg

SEQ ID NO: 46 - DNA, 27 bp, Gallus gallus
  source 1..27: mol_type = genomic DNA
gggagcacagacaccagtaatgatata

SEQ ID NO: 47 - DNA, 369 bp, Gallus gallus
  source 1..369: mol_type = genomic DNA
gccgtgacgttggacgagtccgggggcggcctccagacgcccggaggagggctcagcctcgtctgcaaggcctccgggttcaccttcagaagttacgccatgtactgggtgcgacaggcgcccggcaaggggctggagtggcttgcagggattagtagtagtggtagatacacaggctacgcgccggcggtgaagggccgtgccaccatctcgagggacaacgggcagagcacagtgaggctgcagctgagcaacctcagggctgaggacgccggcacctactactgcgccaaagatgtttacgattcttggacttacgctaatcgtatcgacgcatggggccacgggaccgaagtcatcgtgtcgtcc

SEQ ID NO: 48 - DNA, 318 bp, Gallus gallus
  source 1..318: mol_type = genomic DNA
gcgctgactcagccatcctcggtgtcagcaaacccgggagagaccgtcaagatcacctgctccgggggtggtaggcgcggttactatggctggtaccagcagaagtctcctggcagtgcccctgtcactgtgatctataacaacgacgagagaccctcaaacatcccttcacgattctccggttttaaatccggctccacggccacattaaccatcactggggtccaagccgaggacgaggctgtctattactgtgggagtggagacaccactacggatagtggtatatttggggccgggacaaccctgaccgtccta

SEQ ID NO: 49 - DNA, 390 bp, Gallus gallus
  source 1..390: mol_type = genomic DNA
gccgtgacgttggacgagtccgggggcggcctccagacgcccggaagagcgctcagcctcgtctgcaaggcctccgggttcaccttcagcgattatggcatgggttggatgcgccaggcacccggcaaggggctggaatgggtcggtgctattagcaacagaggtagtcacacatactacggggcggcggtgaagggccgtgccaccatctcgagggacaacgggcagagcacagtgaggctgcagctgaacaacctcagggctgaggacaccggcacctactactgcgccaaagatgctggtacctgtatttccagttacggtttcagttgtgtatctgctgctagcatcgacgcatggggccacgggaccgaagtcatcgtgtcgtcc

SEQ ID NO: 50 - DNA, 330 bp, Gallus gallus
  source 1..330: mol_type = genomic DNA
gcgctgactcagccatcctcggtgtcagcaaacctgggaggaaccgtcaagatcacctgctccgggggtagtggcagctatggtggaagttactattatggctggtaccagcagaaggcacctggcagtgcccctgtcactctgatctatgacaacaccaacagaccctcgaacatcccttcacgattctccggttccaaatccggctccacagccacattaaccatcactggggtccaagccgacgacgaggctgtctatttctgtgggagcatagacagcatcagtgatgctgatatatttggggccgggacaaccctgaccgtccta

SEQ ID NO: 51 - DNA, 351 bp, Gallus gallus
  source 1..351: mol_type = genomic DNA
gccgtgacgttggacgagtccgggggcggcctccagacgcccggaggagcgctcagcctcgtctgcaaggcctccgggttcaccttcacccgttacgccatacagtgggtgcgacaggcgcccggcaaagggctggaatgggtcggtgttattaacagtggtggtcgcacactctacgcgccggcggtgaagggccgtgccaccatctcgagggacaatgggcagagcacagtgaggctgcagctgaacaacctcagggctgaggacaccgccatctactactgcgtcagaggtggttatgcttatggcatcgagacatggggccacgggaccgaagtcatcgtgtcgtcc

SEQ ID NO: 52 - DNA, 306 bp, Gallus gallus
  source 1..306: mol_type = genomic DNA
gcgctgactcagccatcctcggtgtcagcgaacccgggagaaactgtcaagatcacctgctccgggagtaggtatgattatggctggtaccagcagaagtcacctggcagtgcccctgtcactctgatctattacaacaacaagagaccctcggacatcccttcacgattctccggttccaaatccggctccacacacacactaaccatcactggggtccaagccgacgacgaggctgtctatttctgtgggagcacagacaccagtaatgatatatttggggccgggacaaccctgaccgtccta

SEQ ID NO: 53 - DNA, 990 bp, Homo sapiens
  source 1..990: mol_type = genomic DNA
gcctctacaaagggccccagcgtgttccctctggcccctagcagcaagagcacatctggcggaacagccgccctgggctgcctcgtgaaggactactttcccgagcccgtgaccgtgtcctggaactctggcgctctgacaagcggcgtgcacacctttccagccgtgctgcagagcagcggcctgtactctctgagcagcgtcgtgacagtgcccagcagctctctgggcacccagacctacatctgcaacgtgaaccacaagcccagcaacaccaaggtggacaagaaggtggaacccaagagctgcgacaagacccacacctgtcccccttgtcctgcccccgaactgctgggaggcccttccgtgttcctgttccccccaaagcccaaggacaccctgatgatcagccggacccccgaagtgacctgcgtggtggtggatgtgtcccacgaggaccctgaagtgaagttcaattggtacgtggacggcgtggaagtgcacaacgccaagaccaagcctagagaggaacagtacaacagcacctaccgggtggtgtccgtgctgacagtgctgcaccaggactggctgaacggcaaagagtacaagtgcaaggtgtccaacaaggccctgcctgcccccatcgagaaaaccatcagcaaggccaagggccagccccgcgaaccccaggtgtacacactgcccccaagcagggacgagctgaccaagaaccaggtgtccctgacctgtctcgtgaaaggcttctacccctccgatatcgccgtggaatgggagagcaacggccagcccgagaacaactacaagaccaccccccctgtgctggacagcgacggctcattcttcctgtacagcaagctgaccgtggacaagtcccggtggcagcagggcaacgtgttcagctgcagcgtgatgcacgaggccctgcacaaccactacacccagaagtccctgagcctgagccccggcaaa

SEQ ID NO: 54 - DNA, 315 bp, Homo sapiens
  source 1..315: mol_type = genomic DNA
ggtcagcccaaggctgccccctcggtcactctgttcccgccctcctctgaggagcttcaagccaacaaggccacactggtgtgtctcataagtgacttctacccgggagccgtgacagtggcctggaaggcagatagcagccccgtcaaggcgggagtggagaccaccacaccctccaaacaaagcaacaacaagtacgcggccagcagctatctgagcctgacgcctgagcagtggaagtcccacagaagctacagctgccaggtcacgcatgaagggagcaccgtggagaagacagtggcccctacagaatgt